European Patent Specification EP 3 775 222 B1, published January 3, 2024. Title: Fungal chaperone proteins. Applicant: Novozymes A/S. The sequence listing filed with the application follows.

SEQUENCE LISTING (25 sequences)

SEQ ID NO: 1 - DNA, 2044 bp, Aspergillus oryzae
atggcccccgctgtcggtatcgatttgggtaccacctactcctgtgtgggtgtgttccgtgatgaccgcattgaaatcattgccaacgaccagggtaaccgtaccaccccttccttcgtggctttcaccgataccgagcgtctcatcggtgatgccgccaagaaccaggtcgcaatgaaccctcacaacactgtcttcgatgccaagcgtctgatcggtcgtcgttatgccgatgctgaggtccagtctgatatgaagcactggcccttcaagatcgtcgataagggtggcaagcccatcatccaggttgagttcaagggcgaagagaagcaattcactcccgaggaagtctcctctatggtcctgaccaagatgcgtgagaccgcagaggcctatcttggtggtactgttaacaacgccgttatcactgtccccgcctacttcaacgactcccagcgtcaggctaccaaggatgctggtctcatcgccggtctgaacgtcctccgtatcattaacgagcccactgccgccgccatcgcctacggtctagacaagaaggccgagggcgagcgcaatgtcctgatcttcgatttgggtggtggtacctttgatgtttctctcttgaccattgaagaaggtatcttcgaggtcaaggctaccgctggtgacactcaccttggtggtgaggacttcgacaaccgtctcgtcaaccatttcgttaacgagttcaaacgcaagcacaagaaaggttggtcttttgattccgataatcgcaaagcccccaatgctaacttggatatgacagatctcactaccaacgcgcgtgccctccgccgtctccgcactgcctgtgagcgtgccaagcgtacactgtcttctgctgcccagacctctattgaaatcgactctctctttgagggtattgatttctatacctcgatcacccgtgcccgtttcgaggaactttgccaggacctcttccgcggtactatggagcctgtcgagcgtgtcctccgtgatgccaagatcgacaagtcctctgtccacgagattgtcctggtcggtggctctacccgtatccccaagatccagcgccttgtctccgattttttcaacaaggagcccaacaagtccatcaaccccgatgaggccgttgcctacggtgctgccgttcaggctgccatcctgtccggtgatagttcctccaagtccaccaacgagatcctgctactcgacgttgcccccctgtctctcggtatcgaaaccgctggtggtgtcatgaccgctctaatcaagcgcaacaccacaattcccaccaagaagtccgagactttctccacttactctgacaaccagcctggtgtgttgatccaggtttacgagggtgaacgtgctcgtactaaggacaacaacctgctcggaaagttcgagctcactggcattcctcccgctccccgtggtgttcctcagatcgaggttaccttcgatgtcgatgccaacggtatcatgaacgtttctgccgtcgagaagggcactggaaagaccaacaagatcaccatcaccaacgacaagggccgtctctccaaggaggagattgagcgcatgcttgccgatgccgagaagtacaaggctgaggatgaggctgaggcttcccgtatccaggccaagaacggccttgagtcttatgcctactccctcaagaacaccatcagcgagggcaagcttaccatctctgactccgacaaggagaaggtcaccagcaaggttgatgagatcatcggttggcttgacagcaaccagaccgccaccaaggaggagtacgagtctcagcagaaggagctcgaagggtatgtgatatgaaaccccttttatccctccatgactaatatgatgctaactgtgcgctagtgttgccaaccctatcatctccgctgcttatggcggtgccgctggtgctgctcctggcggtgctcccggcgctgcccccggtggctccactcgcaccgctgacgaggttgaggagaagcccgaggagcttgactaa

SEQ ID NO: 2 - protein, 641 aa, Aspergillus oryzae
MAPAVGIDLGTTYSCVGVFRDDRIEIIANDQGNRTTPSFVAFTDTERLIGDAAKNQVAMNPHNTVFDAKRLIGRRYADAEVQSDMKHWPFKIVDKGGKPIIQVEFKGEEKQFTPEEVSSMVLTKMRETAEAYLGGTVNNAVITVPAYFNDSQRQATKDAGLIAGLNVLRIINEPTAAAIAYGLDKKAEGERNVLIFDLGGGTFDVSLLTIEEGIFEVKATAGDTHLGGEDFDNRLVNHFVNEFKRKHKKDLTTNARALRRLRTACERAKRTLSSAAQTSIEIDSLFEGIDFYTSITRARFEELCQDLFRGTMEPVERVLRDAKIDKSSVHEIVLVGGSTRIPKIQRLVSDFFNKEPNKSINPDEAVAYGAAVQAAILSGDSSSKSTNEILLLDVAPLSLGIETAGGVMTALIKRNTTIPTKKSETFSTYSDNQPGVLIQVYEGERARTKDNNLLGKFELTGIPPAPRGVPQIEVTFDVDANGIMNVSAVEKGTGKTNKITITNDKGRLSKEEIERMLADAEKYKAEDEAEASRIQAKNGLESYAYSLKNTISEGKLTISDSDKEKVTSKVDEIIGWLDSNQTATKEEYESQQKELEGVANPIISAAYGGAAGAAPGGAPGAAPGGSTRTADEVEEKPEELD

SEQ ID NO: 3 - DNA, 2495 bp, Aspergillus oryzae
atgagtgtagttggaatcgacttcggtgcccagagcaccaagattggtgtcgcccgtaataagggtatcgacattgtgcgtatcatgccttccccaccttcagcgcttccctatacttttttttttcttaccaaccccgtcacttgaaccattttgaaatgcaaagactaaccgtcggtgcgactcaatttagatcaccaacgaagtttccaacagatctactccgtatgtccacccctctgttaagattccgccccaccccagccaacaacgagcttaacggcgtgggttttatctagccatcctatactgactgtgtgtgatgttcagctccctcatctccttcgacaacaaatgtagatatctcggtgaggctgctaagacacgagagacctccaacctgaagaacactgttgcaaacctcaagcgcctgattggccgctcattcagcgaccctgatgttcagatcgagcagagcttcaatactgctactctctgcgatgtgaacggccaggctggtgtcgaggttaacttccgtcagcagaagcagaagttctcggctactcagctggtcgccatgtacctgaccaagatcagagatactgccgccaacgaactgcaaatccccgtctccgatgtcaccatcagcgttcccgcctggttcaccgatgttcagcgccgggccatgcttgacgctggtgagattgctggtctcaaggttctgagactgatcaacgacaccaccgccaccgctcttggatatggtatcactaagctcgatctccccggtcccgaggagaagcctcgccgcgtcatgttcgttgatatcggccacagcgactacaccgcttcgattgttgagttccgcaagggtgaactaaacgtcaaggctaccgcctgcgaccgccacttcggtggccgtaacttcgaccttgccctcactgagcatttcgccgaggagttcaaggagaagttcaagatcgacgttcgtaagaacgccaaggcttgggctcgtaccctcgctgccgctgagaagatgaagaaggtcctttcggcgaaccctgctgcccccatgagcatcgaatccctgatggaggacgtcgatgtccgcgccattgtcaagcgtgaggagctggagaccatggttcagcctctcctggagcgcgtccttgttcccatcgagcaggccctcgccgaggccaagctcaagcccgaggatattgacagcattgagatggttggtggctgcactcgtgtcccctccatcaaggaggccgtttccaagttcttcggcaagaacctttccttcaccctgaaccaagatgaggccatcgctcgcggttgtgccttcagctgtgccatcctctcccccgtcttccgtgtccgtgacttctccgtgcacgacatcgtcaactaccccatcgagttcacctgggagcagtccgcagatatccccgacgaggacaccagcctgaccgtcttcggtcgcggcaatgtcatgccctcgaccaagattctcacgttctaccgcaagcagcctttcgatctcgaagctcgttacgctagccccgaggagcttcctggaaagaccgacccctgggtgggccgcttctctgtcaagggtgtcaaggccgatgccaacgatgacttcatgatttgcaagctcaaggcccgcctgaacttgcacggtatcctcaacgttgagtctggttactacgtcgaggacatggaagtggaggagcctgtcgaggaggatgctgatgtgagttggattcgtatcgtaatgcgcgcagcttttgttactaacatgcgactaggctatggacaccgatgctaagggtgatgagcagcccaagaagacccgcaaggtcaagaagcaggttcgcaagggcgacctgcccattgtcgccggcacccctgccattgagccttccgtcaaggaagcctggatcgaaggcgagaaggccatgtatctgcatgataagactatcgccgagaccgacgagaagaagaacgagcttgaaaccacgatttacgatatgcgtgacaggaaatatggtcgctacgccagattcctcgaagatgaggcgaagaagcaggccttcgatgacaagctggatgagctcgaggtatgttcactctccttttctagccagatcgccgtgtctgtcaaggttttgtgctcgtgctaaccacgattttagaactggctgtatgatgatgagggcggtgctgacaccactctcgatgtctatgctggcaagctccaggagatcaagaagctggtgcagccattcgaggagacccttgaggacgagcgccagcaagctctggctgaagagctcgctaagaagcgcgctgaggaagaagccaagcgcgcggctgaagagcaggccaagaaggccgcggccgctgctatgaactttgaagagagaaatgagacgatgcctgatgctcctgctcaggaggaagcccccgctggcgacaagcagtaa

SEQ ID NO: 4 - protein, 713 aa, Aspergillus oryzae
MSVVGIDFGAQSTKIGVARNKGIDIITNEVSNRSTPSLISFDNKCRYLGEAAKTRETSNLKNTVANLKRLIGRSFSDPDVQIEQSFNTATLCDVNGQAGVEVNFRQQKQKFSATQLVAMYLTKIRDTAANELQIPVSDVTISVPAWFTDVQRRAMLDAGEIAGLKVLRLINDTTATALGYGITKLDLPGPEEKPRRVMFVDIGHSDYTASIVEFRKGELNVKATACDRHFGGRNFDLALTEHFAEEFKEKFKIDVRKNAKAWARTLAAAEKMKKVLSANPAAPMSIESLMEDVDVRAIVKREELETMVQPLLERVLVPIEQALAEAKLKPEDIDSIEMVGGCTRVPSIKEAVSKFFGKNLSFTLNQDEAIARGCAFSCAILSPVFRVRDFSVHDIVNYPIEFTWEQSADIPDEDTSLTVFGRGNVMPSTKILTFYRKQPFDLEARYASPEELPGKTDPWVGRFSVKGVKADANDDFMICKLKARLNLHGILNVESGYYVEDMEVEEPVEEDADAMDTDAKGDEQPKKTRKVKKQVRKGDLPIVAGTPAIEPSVKEAWIEGEKAMYLHDKTIAETDEKKNELETTIYDMRDRKYGRYARFLEDEAKKQAFDDKLDELENWLYDDEGGADTTLDVYAGKLQEIKKLVQPFEETLEDERQQALAEELAKKRAEEEAKRAAEEQAKKAAAAAMNFEERNETMPDAPAQEEAPAGDKQ

SEQ ID NO: 5 - DNA, 2173 bp, Aspergillus oryzae
atgtccgagacttttgagttccaggctgagatctctcagctcctttctcttatcatcaacactgtctactccaacaaggagattttcctgcgtgaacttatctccaatgcctccgatgcccttgacaagatccgctatgagtctttgtcggacccttccaagctcgactcaggcaaggacctccgtatcgatatcattcccaacaaggaggccaagaccttgactatccgtgataccggtatcggtatgaccaaggctgtaagtcaatctcgtctcggttgccattatatgtctacacagaccccaatctaatcatatcgcttttgtataggacctgatcaacaaccttggtaccatcgctcgctctggtaccaagcagttcatggaagccctctccgcaggtgccgatatttccatgattggccagttcggtgttggcttctactctgcttaccttgtcgctgaccgcgtcactgtcatctctaagcacaacgatgatgagcagtacgtctgggagtccgctgccggcggtaccttcacgctcacccaggacaccgagggtgagccccttggccgtggtaccaagatgatccttcacttgaaggatgagcagaccgactacctcaacgagagccgcatcaaggaggttgttcgcaagcactccgaattcatctcttaccccatctacctccacgttctgaaggaaaccgagaaggaggttcctgatgaggaggaagagaccaaggaagaggaaggcgatgagaaaaagcccaaaattgaggaggttgacgaagaagaagaaaagaaggagaagaagaccaagactgtcaaggagagcaagatcgaggaggaggagctcaacaagactaagcccatctggacccgtaaccctgctgatatcactcaggaggaatacgctgccttctacaagtctctctccaatgactgggaggatcaccttgccgtcaagcacttctccgttgagggtcagctcgagttccgtgccatcctctatattcctaagcgtgctcctttcgacctcttcgagaccaagaagactaagaacaacatcaagctctatgttcgccgtgtcttcatcaccgacgacgccaccgacctcatccctgagtggctcagcttcatcaagggtgttgttgattcagaggaccttcctctcaacttgtcccgtgagaccctgcagcagaacaagatcatgaaggttatcaaaaagaacattgtcaagaagacccttgagctcttcaccgagattgctgaagaccgtgagcagtttgacaagttctactccgccttcagcaagaacatcaaacttggtgtccacgaggatgctcagaaccgccagactctcgctaagctgctccgttaccagtccaccaagtcgggtgatgaggtcacctccctctctgactatgtcacccgcatgcctgagcaccagaagcaaatctactacatcactggcgagtctatcaaggctgtcgccaagtctcctttccttgacagcctcaagcagaagaactttgaggttctcttcctggttgaccctattgatgagtacgctttcactcagcttaaggagtttgatggcaagaagcttgtcgacatcactaaggacttcgaactcgaggagtccgaggaggagaaggctgagcgtgagaaggaggagaaggagttcgagggcctcgccaagagccttaagaacatcctcggtgacaaggttgagaaggttgttgtctctcacaaacttgttggctctccttgcgccatccgtactggccagtttggttggtctgccaatatggagcgtatcatgaaggcccaggccctccgtgacacctccatgagctcctacatgtcttccaagaagaccttcgagatctctcccaagtctgctatcatcaaggagctcaagaagaaggtcgaggctgatggtgaaagcgaccgtaccgtcaagtccatcactcagcttctgttcgagacctctcttttggtttccggcttcaccatcgacgagcctgccagctttgccgagcgcatccacaagcttgtgtctcttggtctgaacgtcgacgaggaggctgagacctctgaggaaaaggccgctgaggaggctcctgccgctgccaccggtgagagctccatggaggaggttgactaa

SEQ ID NO: 6 - protein, 699 aa, Aspergillus oryzae
MSETFEFQAEISQLLSLIINTVYSNKEIFLRELISNASDALDKIRYESLSDPSKLDSGKDLRIDIIPNKEAKTLTIRDTGIGMTKADLINNLGTIARSGTKQFMEALSAGADISMIGQFGVGFYSAYLVADRVTVISKHNDDEQYVWESAAGGTFTLTQDTEGEPLGRGTKMILHLKDEQTDYLNESRIKEVVRKHSEFISYPIYLHVLKETEKEVPDEEEETKEEEGDEKKPKIEEVDEEEEKKEKKTKTVKESKIEEEELNKTKPIWTRNPADITQEEYAAFYKSLSNDWEDHLAVKHFSVEGQLEFRAILYIPKRAPFDLFETKKTKNNIKLYVRRVFITDDATDLIPEWLSFIKGVVDSEDLPLNLSRETLQQNKIMKVIKKNIVKKTLELFTEIAEDREQFDKFYSAFSKNIKLGVHEDAQNRQTLAKLLRYQSTKSGDEVTSLSDYVTRMPEHQKQIYYITGESIKAVAKSPFLDSLKQKNFEVLFLVDPIDEYAFTQLKEFDGKKLVDITKDFELEESEEEKAEREKEEKEFEGLAKSLKNILGDKVEKVVVSHKLVGSPCAIRTGQFGWSANMERIMKAQALRDTSMSSYMSSKKTFEISPKSAIIKELKKKVEADGESDRTVKSITQLLFETSLLVSGFTIDEPASFAERIHKLVSLGLNVDEEAETSEEKAAEEAPAAATGESSMEEVD

SEQ ID NO: 7 - DNA, 34 bp, Artificial Sequence
  Primer oAT3702
ccattgtgcctgtggggtttattgttcagagaag

SEQ ID NO: 8 - DNA, 22 bp, Artificial Sequence
  Primer oAT3703
ccacaggcacaatggcccccgc

SEQ ID NO: 9 - DNA, 36 bp, Artificial Sequence
  Primer oAT3704
tgtcagtgtgaaccgacgtagcctgttttgaattcc

SEQ ID NO: 10 - DNA, 30 bp, Artificial Sequence
  Primer oAT3705
cggttcacactgacagaggatggagttctg

SEQ ID NO: 11 - DNA, 32 bp, Artificial Sequence
  Primer oAT3706
cccacaggcatcatgtccgagacttttgagtt

SEQ ID NO: 12 - DNA, 52 bp, Artificial Sequence
  Primer oAT3707
cgatcatcgagaattccatggtgttttgatcattttaaatttttatatggcg

SEQ ID NO: 13 - DNA, 33 bp, Artificial Sequence
  Primer oAT3708
catgatgcctgtggggtttattgttcagagaag

SEQ ID NO: 14 - DNA, 53 bp, Artificial Sequence
  Primer oAT3709
ccgcggccgcgaattccatggtgttttgatcattttaaatttttatatggcgg

SEQ ID NO: 15 - DNA, 38 bp, Artificial Sequence
  Primer oAT3713
tgagagtgcaccatagatctgtaggagtgagtacccgg

SEQ ID NO: 16 - DNA, 36 bp, Artificial Sequence
  Primer oAT3714
gccattgtggctctgtttagatgtgtctatgtggcg

SEQ ID NO: 17 - DNA, 23 bp, Artificial Sequence
  Primer oAT3715
acagagccacaatggcccccgct

SEQ ID NO: 18 - DNA, 32 bp, Artificial Sequence
  Primer oAT3716
aacagagcatgtccgagacttttgagttccag

SEQ ID NO: 19 - DNA, 35 bp, Artificial Sequence
  Primer oAT3717
ctcggacatgctctgtttagatgtgtctatgtggc

SEQ ID NO: 20 - DNA, 38 bp, Artificial Sequence
  Primer oAT3718
cgatcatcgagaattgatctgtaggagtgagtacccgg

SEQ ID NO: 21 - DNA, 30 bp, Artificial Sequence
  Primer oAT3719
cggttcacactgacacaactgaatgcgccc

SEQ ID NO: 22 - DNA, 32 bp, Artificial Sequence
  Primer oAT3720
cccacaggcatcatgagtgtagttggaatcga

SEQ ID NO: 23 - DNA, 52 bp, Artificial Sequence
  Primer oAT3725
tcactcctacagatccatggtgttttgatcattttaaatttttatatggcgg

SEQ ID NO: 24 - DNA, 38 bp, Artificial Sequence
  Primer oAT3726
gatcaaaacaccatggatctgtaggagtgagtacccgg

SEQ ID NO: 25 - DNA, 30 bp, Artificial Sequence
  Primer oAT3727
gatcatcgagaattcgaggatggagttctg